European Patent Specification EP 3 204 414 B1, published December 4, 2024. Title: NOVEL ANTI-NODAL ANTIBODIES AND METHODS OF USING SAME. Applicant: ANN AND ROBERT H. LURIE CHILDREN'S HOSPITAL OF CHICAGO RUVO, MENOTTI SANDOMENICO, ANNAMARIA LEONARDI, ANTONIO SANGUIGNO, LUCA. The sequence listing filed with the application follows.

SEQUENCE LISTING (32 sequences)

SEQ ID NO: 1 - protein, 110 aa, Artificial Sequence
  Synthetic
DIKMTQSPASLSASVGETVTITCRASGNIHNYLAWYQQKQGKSPQLLVYNAKTLADGVPSRFSGSGSGTQYSLKINSLQPEDFGSYYCQHFWSTPHVRCWDQAGTETEAW

SEQ ID NO: 2 - protein, 122 aa, Artificial Sequence
  Synthetic
  misc_feature (120)..(120): Xaa can be any naturally occurring amino acid
VKLVESGGGLVKPGGSLKLSCAASGFTFSSYAMSWVRQTPEKRLEWVASISSGGCTYYPDSVKGRFTISRDNARNILYLQMSSLRSEDTAMYYCARGSMITADGNSLLLCYGLLGSRNLXHR

SEQ ID NO: 3 - protein, 111 aa, Artificial Sequence
  Synthetic
VKLVESGGGLVQPGGSMKLSCVASGFTFRNYWMSWVRQSPEKGLEWVAEIRLKSDNYAARYAESVKGKFTISRDDSKSRLYLQMNSLRAEDTGIYYCTGIRRFAYWGQGTL

SEQ ID NO: 4 - protein, 8 aa, Artificial Sequence
  Synthetic
GNIHNYLA

SEQ ID NO: 5 - protein, 11 aa, Artificial Sequence
  Synthetic
LLVYNAKTLAD

SEQ ID NO: 6 - protein, 15 aa, Artificial Sequence
  Synthetic
QHFWSTPHVRCWDQA

SEQ ID NO: 7 - protein, 9 aa, Artificial Sequence
  Synthetic
FTFSSYAMS

SEQ ID NO: 8 - protein, 13 aa, Artificial Sequence
  Synthetic
WVASISSGGCTYY

SEQ ID NO: 9 - protein, 11 aa, Artificial Sequence
  Synthetic
ARGSMITADGN

SEQ ID NO: 10 - protein, 9 aa, Artificial Sequence
  Synthetic
FTFRNYWMS

SEQ ID NO: 11 - protein, 16 aa, Artificial Sequence
  Synthetic
WVAEIRLKSDNYAARY

SEQ ID NO: 12 - protein, 7 aa, Artificial Sequence
  Synthetic
GIRRFAY

SEQ ID NO: 13 - protein, 26 aa, Artificial Sequence
  Synthetic
PNPVGEEFHPTNHAYIQSLLKRYQPH

SEQ ID NO: 14 - protein, 26 aa, Artificial Sequence
  Synthetic
PNPVGAAFHPTNHAYIQSLLKRYQPH

SEQ ID NO: 15 - protein, 27 aa, Artificial Sequence
  Synthetic
CPNPVGEEFHPTNHAYIQSLLKRYQPH

SEQ ID NO: 16 - protein, 27 aa, Artificial Sequence
  Synthetic
CPNPVGAAFHPTNHAYIQSLLKRYQPH

SEQ ID NO: 17 - protein, 24 aa, Artificial Sequence
  Synthetic
PNPVGEEFHPTNHAYIQSLLKRYQ

SEQ ID NO: 18 - protein, 25 aa, Artificial Sequence
  Synthetic
CPNPVGEEFHPTNHAYIQSLLKRYQ

SEQ ID NO: 19 - protein, 24 aa, Artificial Sequence
  Synthetic
PNPVGAAFHPTNHAYIQSLLKRYQ

SEQ ID NO: 20 - protein, 24 aa, Artificial Sequence
  Synthetic
PNAAGEEFHPTNHAYIQSLLKRYQ

SEQ ID NO: 21 - protein, 24 aa, Artificial Sequence
  Synthetic
PNPVGEEFHPTNHAAIQSLLKRYQ

SEQ ID NO: 22 - protein, 14 aa, Artificial Sequence
  Synthetic
CPNPVGEEFHPTNH

SEQ ID NO: 23 - protein, 9 aa, Artificial Sequence
  Synthetic
HPTNHAYIQ

SEQ ID NO: 24 - protein, 13 aa, Artificial Sequence
  Synthetic
AYIQSLLKRYQPH

SEQ ID NO: 25 - protein, 13 aa, Artificial Sequence
  Synthetic
PNPVGEEFHPTNH

SEQ ID NO: 26 - protein, 11 aa, Artificial Sequence
  Synthetic
AYIQSLLKRYQ

SEQ ID NO: 27 - protein, 38 aa, Artificial Sequence
  Synthetic
HHLPDRSQLCRKVKFQVDFNLIGWGSWIIYPKQYNAYR

SEQ ID NO: 28 - protein, 37 aa, Artificial Sequence
  Synthetic
CEGECPNPVGEEFHPTNHAYIQSLLKRYQPHRVPSTC

SEQ ID NO: 29 - protein, 35 aa, Artificial Sequence
  Synthetic
CAPVKTKPLSMLYVDNGRVLLDHHKDMIVEECGCL

SEQ ID NO: 30 - protein, 14 aa, Artificial Sequence
  Synthetic
CEFPLRSHLEPTNH

SEQ ID NO: 31 - protein, 14 aa, Artificial Sequence
  Synthetic
CDFPLRSHLEPTNH

SEQ ID NO: 32 - protein, 110 aa, Artificial Sequence
  Synthetic
HHLPDRSQLCRKVKFQVDFNLIGWGSWIIYPKQYNAYRCEGECPNPVGEEFHPTNHAYIQSLLKRYQPHRVPSTCCAPVKTKPLSMLYVDNGRVLLDHHKDMIVEECGCL